European Patent Application EP 4 458 952 A1, published November 6, 2024. Title: CHIMERIC ANTIGEN RECEPTOR-T CELLS TARGETING HIV-INFECTED CELLS. Applicant: Beijing Solobio Genetechnology Co., Ltd. Application CN. The sequence listing filed with the application follows.

SEQUENCE LISTING (50 sequences)

SEQ ID NO: 1 - RNA, 47 nt, synthetic construct
  source 1..47: mol_type = other RNA
atagtaagaatgtatagccttcaagagaggctatacattcttactat

SEQ ID NO: 2 - RNA, 47 nt, synthetic construct
  source 1..47: mol_type = other RNA
tgcttcaagctagtaccagttcaagagactggtactagcttgaagca

SEQ ID NO: 3 - DNA, 47 bp, synthetic construct
  source 1..47: mol_type = other DNA
atagtaagaatgtatagccttcaagagaggctatacattcttactat

SEQ ID NO: 4 - DNA, 47 bp, synthetic construct
  source 1..47: mol_type = other DNA
tgcttcaagctagtaccagttcaagagactggtactagcttgaagca

SEQ ID NO: 5 - RNA, 47 nt, synthetic construct
  source 1..47: mol_type = other RNA
gtgacatagcaggaactacttcaagagagtagttcctgctatgtcac

SEQ ID NO: 6 - RNA, 47 nt, synthetic construct
  source 1..47: mol_type = other RNA
cacaaggctacttccctgattcaagagatcagggaagtagccttgtg

SEQ ID NO: 7 - DNA, 47 bp, synthetic construct
  source 1..47: mol_type = other DNA
gtgacatagcaggaactacttcaagagagtagttcctgctatgtcac

SEQ ID NO: 8 - DNA, 47 bp, synthetic construct
  source 1..47: mol_type = other DNA
cacaaggctacttccctgattcaagagatcagggaagtagccttgtg

SEQ ID NO: 9 - DNA, 215 bp, synthetic construct
  source 1..215: mol_type = other DNA
gaacgctgacgtcatcgacccgctccaaggaatcgcgggcccagtgtcactaggcgggaacacccagcgcgcgtgcgccctggcaggaagatggctgtgagggacaggggagtggcgccctgcaatatttgcatgtcgctatgtgttctgggaaatcaccataaacgtgaaatgtctttggatttgggaatcttataagttctgtatgagaccac

SEQ ID NO: 10 - DNA, 274 bp, synthetic construct
  source 1..274: mol_type = other DNA
gatcctaccaaggtcgggcaggaagagggcctatttcccatgattccttcatatttgcatatacgatacaaggctgttagagagataattagaattaatttgactgtaaacacaaagatattagtacaaaatacgtgacgtagaaagtaataatttcttgggtagtttgcagttttaaaattatgttttaaaatggactatcatatgcttaccgtaacttgaaagtatttcgatttcttggctttatatatcttgtggaaaggacgaaacaccg

SEQ ID NO: 11 - DNA, 73 bp, synthetic construct
  source 1..73: mol_type = other DNA
gcccggatagctcagtcggtagagcacagactttaatctgagggtccagggtcaagtccctgttcgggcgcca

SEQ ID NO: 12 - RNA, 149 nt, synthetic construct
  source 1..149: mol_type = other RNA
gcctgggagagctggggaatttgtacgtaggttccccagctctcccaggcggtggcagtggctccggaggttcaggaagcggcggtagtgggagcgcggagacagcgacgaagagccttcctgtcagagcggagacagcgacgaagagc

SEQ ID NO: 13 - protein, 178 aa, synthetic construct
KKVVLGKKGDTVELTCTASQKKSIQFHWKNSNQIKILGNQGSFLTKGPSKLNDRADSRRSLWDQGNFPLIIKNLKIEDSDTYICEVEDQKEEVQLLVFGLTANSDTHLLQGQSLTLTLESPPGSSPSVQCRSPRGKNIQGGKTLSVSQLELQDSGTWTCTVLQNQKKVEFKIDIVVLA

SEQ ID NO: 14 - protein, 369 aa, synthetic construct
KKVVLGKKGDTVELTCTASQKKSIQFHWKNSNQIKILGNQGSFLTKGPSKLNDRADSRRSLWDQGNFPLIIKNLKIEDSDTYICEVEDQKEEVQLLVFGLTANSDTHLLQGQSLTLTLESPPGSSPSVQCRSPRGKNIQGGKTLSVSQLELQDSGTWTCTVLQNQKKVEFKIDIVVLAFQKASSIVYKKEGEQVEFSFPLAFTVEKLTGSGELWWQAERASSSKSWITFDLKNKEVSVKRVTQDPKLQMGKKLPLHLTLPQALPQYAGSGNLTLALEAKTGKLHQEVNLVVMRATQLQKNLTCEVWGPTSPKLMLSLKLENKEAKVSKREKAVWVLNPEAGMWQCLLSDSGQVLLESNIKVLPTWSTPV

SEQ ID NO: 15 - protein, 249 aa, synthetic construct
DIQMTQSPSSLSASVGDTVTITCQANGYLNWYQQRRGKAPKLLIYDGSKLERGVPSRFSGRRWGQEYNLTINNLQPEDIATYFCQVYEFVVPGTRLDLKRTVAAPGGGGSGGGGSGGGGSQVQLLQSGAAVTKPGASVRVSCEASGYNIRDYFIHWWRQAPGQGLQWVGWINPKTGQPNNPRQFQGRVSLTRHASWDFDTFSFYMDLKALRSDDTAVYFCARQRSDYWDFDVWGSGTQVTVSSASTKGP

SEQ ID NO: 16 - protein, 25 aa, synthetic construct
MNRGVPFRHLLLVLQLALLPAATQG

SEQ ID NO: 17 - protein, 21 aa, synthetic construct
MALPVTALLLPLALLLHAARP

SEQ ID NO: 18 - protein, 28 aa, synthetic construct
IYIWAPLAGTCGVLLLSLVITLYCNHRN

SEQ ID NO: 19 - protein, 67 aa, synthetic construct
KIEVMYPPPYLDNEKSNGTIIHVKGKHLCPSPLFPGPSKPFWVLVVVGGVLACYSLLVTVAFIIFWV

SEQ ID NO: 20 - protein, 58 aa, synthetic construct
AAAFVPVFLPAKPTTTPAPRPPTPAPTIASQPLSLRPEACRPAAGGAVHTRGLDFACD

SEQ ID NO: 21 - protein, 15 aa, synthetic construct
GGGGSGGGGSGGGGS

SEQ ID NO: 22 - protein, 5 aa, synthetic construct
GGGGS

SEQ ID NO: 23 - protein, 112 aa, synthetic construct
RVKFSRSADAPAYQQGQNQLYNELNLGRREEYDVLDKRRGRDPEMGGKPRRKNPQEGLYNELQKDKMAEAYSEIGMKGERRRGKGHDGLYQGLSTATKDTYDALHMQALPPR

SEQ ID NO: 24 - protein, 42 aa, synthetic construct
KRGRKKLLYIFKQPFMRPVQTTQEEDGCSCRFPEEEEGGCEL

SEQ ID NO: 25 - protein, 41 aa, synthetic construct
RSKRSRLLHSDYMNMTPRRPGPTRKHYQPYAPPRDFAAYRS

SEQ ID NO: 26 - protein, 23 aa, synthetic construct
LCARPRRSPAQDGKVYINMPGRG

SEQ ID NO: 27 - protein, 120 aa, synthetic construct
WRRKRKEKQSETSPKEFLTIYEDVKDLKTRRNHEQEQTFPGGGSTIYSMIQSQSSAPTSQEPAYTLYSLIQPSRKSGSRKRNHSPSFNSTIYEVIGKSQPKAQNPARLSRKELENFDVYS

SEQ ID NO: 28 - protein, 154 aa, synthetic construct
KRGRKKLLYIFKQPFMRPVQTTQEEDGCSCRFPEEEEGGCELRVKFSRSADAPAYQQGQNQLYNELNLGRREEYDVLDKRRGRDPEMGGKPRRKNPQEGLYNELQKDKMAEAYSEIGMKGERRRGKGHDGLYQGLSTATKDTYDALHMQALPPR

SEQ ID NO: 29 - protein, 205 aa, synthetic construct
RSKRSRLLHSDYMNMTPRRPGPTRKHYQPYAPPRDFAAYRSGGGGSKRGRKKLLYIFKQPFMRPVQTTQEEDGCSCRFPEEEEGGCELGGGGSRVKFSRSADAPAYQQGQNQLYNELNLGRREEYDVLDKRRGRDPEMGGKPRRKNPQEGLYNELQKDKMAEAYSEIGMKGERRRGKGHDGLYQGLSTATKDTYDALHMQALPPR

SEQ ID NO: 30 - protein, 177 aa, synthetic construct
KRGRKKLLYIFKQPFMRPVQTTQEEDGCSCRFPEEEEGGCELRVKFSRSADAPAYQQGQNQLYNELNLGRREEYDVLDKRRGRDPEMGGKPRRKNPQEGLYNELQKDKMAEAYSEIGMKGERRRGKGHDGLYQGLSTATKDTYDALHMQALPPRLCARPRRSPAQDGKVYINMPGRG

SEQ ID NO: 31 - protein, 176 aa, synthetic construct
RSKRSRLLHSDYMNMTPRRPGPTRKHYQPYAPPRDFAAYRSLCARPRRSPAQDGKVYINMPGRGRVKFSRSADAPAYQQGQNQLYNELNLGRREEYDVLDKRRGRDPEMGGKPRRKNPQEGLYNELQKDKMAEAYSEIGMKGERRRGKGHDGLYQGLSTATKDTYDALHMQALPPR

SEQ ID NO: 32 - protein, 255 aa, synthetic construct
WRRKRKEKQSETSPKEFLTIYEDVKDLKTRRNHEQEQTFPGGGSTIYSMIQSQSSAPTSQEPAYTLYSLIQPSRKSGSRKRNHSPSFNSTIYEVIGKSQPKAQNPARLSRKELENFDVYSLCARPRRSPAQDGKVYINMPGRGRVKFSRSADAPAYQQGQNQLYNELNLGRREEYDVLDKRRGRDPEMGGKPRRKNPQEGLYNELQKDKMAEAYSEIGMKGERRRGKGHDGLYQGLSTATKDTYDALHMQALPPR

SEQ ID NO: 33 - protein, 274 aa, synthetic construct
KRGRKKLLYIFKQPFMRPVQTTQEEDGCSCRFPEEEEGGCELWRRKRKEKQSETSPKEFLTIYEDVKDLKTRRNHEQEQTFPGGGSTIYSMIQSQSSAPTSQEPAYTLYSLIQPSRKSGSRKRNHSPSFNSTIYEVIGKSQPKAQNPARLSRKELENFDVYSRVKFSRSADAPAYQQGQNQLYNELNLGRREEYDVLDKRRGRDPEMGGKPRRKNPQEGLYNELQKDKMAEAYSEIGMKGERRRGKGHDGLYQGLSTATKDTYDALHMQALPPR

SEQ ID NO: 34 - protein, 144 aa, synthetic construct
RSKRSRLLHSDYMNMTPRRPGPTRKHYQPYAPPRDFAAYRSRVKFSRSADAPAYQQGQNQLYNELNLGRREEYDVLDKRRGRDPEMGGKPRRKNPQEGLYNELQKDKMAEAYSEIGMKGERRRGKGHDGLYQGLSTATKDTYDA

SEQ ID NO: 35 - protein, 418 aa, synthetic construct
KKVVLGKKGDTVELTCTASQKKSIQFHWKNSNQIKILGNQGSFLTKGPSKLNDRADSRRSLWDQGNFPLIIKNLKIEDSDTYICEVEDQKEEVQLLVFGLTANSDTHLLQGQSLTLTLESPPGSSPSVQCRSPRGKNIQGGKTLSVSQLELQDSGTWTCTVLQNQKKVEFKIDIVVLAAAAFVPVFLPAKPTTTPAPRPPTPAPTIASQPLSLRPEACRPAAGGAVHTRGLDFACDIYIWAPLAGTCGVLLLSLVITLYCNHRNKRGRKKLLYIFKQPFMRPVQTTQEEDGCSCRFPEEEEGGCELRVKFSRSADAPAYQQGQNQLYNELNLGRREEYDVLDKRRGRDPEMGGKPRRKNPQEGLYNELQKDKMAEAYSEIGMKGERRRGKGHDGLYQGLSTATKDTYDALHMQALPPR

SEQ ID NO: 36 - protein, 469 aa, synthetic construct
KKVVLGKKGDTVELTCTASQKKSIQFHWKNSNQIKILGNQGSFLTKGPSKLNDRADSRRSLWDQGNFPLIIKNLKIEDSDTYICEVEDQKEEVQLLVFGLTANSDTHLLQGQSLTLTLESPPGSSPSVQCRSPRGKNIQGGKTLSVSQLELQDSGTWTCTVLQNQKKVEFKIDIVVLAAAAFVPVFLPAKPTTTPAPRPPTPAPTIASQPLSLRPEACRPAAGGAVHTRGLDFACDIYIWAPLAGTCGVLLLSLVITLYCNHRNRSKRSRLLHSDYMNMTPRRPGPTRKHYQPYAPPRDFAAYRSGGGGSKRGRKKLLYIFKQPFMRPVQTTQEEDGCSCRFPEEEEGGCELGGGGSRVKFSRSADAPAYQQGQNQLYNELNLGRREEYDVLDKRRGRDPEMGGKPRRKNPQEGLYNELQKDKMAEAYSEIGMKGERRRGKGHDGLYQGLSTATKDTYDALHMQALPPR

SEQ ID NO: 37 - protein, 432 aa, synthetic construct
KKVVLGKKGDTVELTCTASQKKSIQFHWKNSNQIKILGNQGSFLTKGPSKLNDRADSRRSLWDQGNFPLIIKNLKIEDSDTYICEVEDQKEEVQLLVFGLTANSDTHLLQGQSLTLTLESPPGSSPSVQCRSPRGKNIQGGKTLSVSQLELQDSGTWTCTVLQNQKKVEFKIDIVVLAGGGGSGGGGSGGGGSFPGPSKPFWVLVVVGGVLACYSLLVTVAFIIFWVRSKRSRLLHSDYMNMTPRRPGPTRKHYQPYAPPRDFAAYRSGGGGSKRGRKKLLYIFKQPFMRPVQTTQEEDGCSCRFPEEEEGGCELGGGGSRVKFSRSADAPAYQQGQNQLYNELNLGRREEYDVLDKRRGRDPEMGGKPRRKNPQEGLYNELQKDKMAEAYSEIGMKGERRRGKGHDGLYQGLSTATKDTYDALHMQALPPR

SEQ ID NO: 38 - protein, 547 aa, synthetic construct
KKVVLGKKGDTVELTCTASQKKSIQFHWKNSNQIKILGNQGSFLTKGPSKLNDRADSRRSLWDQGNFPLIIKNLKIEDSDTYICEVEDQKEEVQLLVFGLTANSDTHLLQGQSLTLTLESPPGSSPSVQCRSPRGKNIQGGKTLSVSQLELQDSGTWTCTVLQNQKKVEFKIDIVVLAFQKASSIVYKKEGEQVEFSFPLAFTVEKLTGSGELWWQAERASSSKSWITFDLKNKEVSVKRVTQDPKLQMGKKLPLHLTLPQALPQYAGSGNLTLALEAKTGKLHQEVNLVVMRATQLQKNLTCEVWGPTSPKLMLSLKLENKEAKVSKREKAVWVLNPEAGMWQCLLSDSGQVLLESNIKVLPTWSTPVQPMALIVLGGVAGLLLFIGLGIFFKRGRKKLLYIFKQPFMRPVQTTQEEDGCSCRFPEEEEGGCELRVKFSRSADAPAYQQGQNQLYNELNLGRREEYDVLDKRRGRDPEMGGKPRRKNPQEGLYNELQKDKMAEAYSEIGMKGERRRGKGHDGLYQGLSTATKDTYDALHMQALPPR

SEQ ID NO: 39 - protein, 489 aa, synthetic construct
DIQMTQSPSSLSASVGDTVTITCQANGYLNWYQQRRGKAPKLLIYDGSKLERGVPSRFSGRRWGQEYNLTINNLQPEDIATYFCQVYEFVVPGTRLDLKRTVAAPGGGGSGGGGSGGGGSQVQLLQSGAAVTKPGASVRVSCEASGYNIRDYFIHWWRQAPGQGLQWVGWINPKTGQPNNPRQFQGRVSLTRHASWDFDTFSFYMDLKALRSDDTAVYFCARQRSDYWDFDVWGSGTQVTVSSASTKGPAAAFVPVFLPAKPTTTPAPRPPTPAPTIASQPLSLRPEACRPAAGGAVHTRGLDFACDIYIWAPLAGTCGVLLLSLVITLYCNHRNKRGRKKLLYIFKQPFMRPVQTTQEEDGCSCRFPEEEEGGCELRVKFSRSADAPAYQQGQNQLYNELNLGRREEYDVLDKRRGRDPEMGGKPRRKNPQEGLYNELQKDKMAEAYSEIGMKGERRRGKGHDGLYQGLSTATKDTYDALHMQALPPR

SEQ ID NO: 40 - protein, 540 aa, synthetic construct
DIQMTQSPSSLSASVGDTVTITCQANGYLNWYQQRRGKAPKLLIYDGSKLERGVPSRFSGRRWGQEYNLTINNLQPEDIATYFCQVYEFVVPGTRLDLKRTVAAPGGGGSGGGGSGGGGSQVQLLQSGAAVTKPGASVRVSCEASGYNIRDYFIHWWRQAPGQGLQWVGWINPKTGQPNNPRQFQGRVSLTRHASWDFDTFSFYMDLKALRSDDTAVYFCARQRSDYWDFDVWGSGTQVTVSSASTKGPAAAFVPVFLPAKPTTTPAPRPPTPAPTIASQPLSLRPEACRPAAGGAVHTRGLDFACDIYIWAPLAGTCGVLLLSLVITLYCNHRNRSKRSRLLHSDYMNMTPRRPGPTRKHYQPYAPPRDFAAYRSGGGGSKRGRKKLLYIFKQPFMRPVQTTQEEDGCSCRFPEEEEGGCELGGGGSRVKFSRSADAPAYQQGQNQLYNELNLGRREEYDVLDKRRGRDPEMGGKPRRKNPQEGLYNELQKDKMAEAYSEIGMKGERRRGKGHDGLYQGLSTATKDTYDALHMQALPPR

SEQ ID NO: 41 - protein, 582 aa, synthetic construct
KKVVLGKKGDTVELTCTASQKKSIQFHWKNSNQIKILGNQGSFLTKGPSKLNDRADSRRSLWDQGNFPLIIKNLKIEDSDTYICEVEDQKEEVQLLVFGLTANSDTHLLQGQSLTLTLESPPGSSPSVQCRSPRGKNIQGGKTLSVSQLELQDSGTWTCTVLQNQKKVEFKIDIVVLAFQKASSIVYKKEGEQVEFSFPLAFTVEKLTGSGELWWQAERASSSKSWITFDLKNKEVSVKRVTQDPKLQMGKKLPLHLTLPQALPQYAGSGNLTLALEAKTGKLHQEVNLVVMRATQLQKNLTCEVWGPTSPKLMLSLKLENKEAKVSKREKAVWVLNPEAGMWQCLLSDSGQVLLESNIKVLPTWSTPVPRKIEVMYPPPYLDNEKSNGTIIHVKGKHLCPSPLFPGPSKPFWVLVVVGGVLACYSLLVTVAFIIFWVRSKRSRLLHSDYMNMTPRRPGPTRKHYQPYAPPRDFAAYRSRVKFSRSADAPAYQQGQNQLYNELNLGRREEYDVLDKRRGRDPEMGGKPRRKNPQEGLYNELQKDKMAEAYSEIGMKGERRRGKGHDGLYQGLSTATKDTYDA

SEQ ID NO: 42 - protein, 306 aa, synthetic construct
KKVVLGKKGDTVELTCTASQKKSIQFHWKNSNQIKILGNQGSFLTKGPSKLNDRADSRRSLWDQGNFPLIIKNLKIEDSDTYICEVEDQKEEVQLLVFGLTANSDTHLLQGQSLTLTLESPPGSSPSVQCRSPRGKNIQGGKTLSVSQLELQDSGTWTCTVLQNQKKVEFKIDIVVLAAAAFVPVFLPAKPTTTPAPRPPTPAPTIASQPLSLRPEACRPAAGGAVHTRGLDFACDIYIWAPLAGTCGVLLLSLVITLYCNHRNKRGRKKLLYIFKQPFMRPVQTTQEEDGCSCRFPEEEEGGCEL

SEQ ID NO: 43 - protein, 441 aa, synthetic construct
KKVVLGKKGDTVELTCTASQKKSIQFHWKNSNQIKILGNQGSFLTKGPSKLNDRADSRRSLWDQGNFPLIIKNLKIEDSDTYICEVEDQKEEVQLLVFGLTANSDTHLLQGQSLTLTLESPPGSSPSVQCRSPRGKNIQGGKTLSVSQLELQDSGTWTCTVLQNQKKVEFKIDIVVLAAAAFVPVFLPAKPTTTPAPRPPTPAPTIASQPLSLRPEACRPAAGGAVHTRGLDFACDIYIWAPLAGTCGVLLLSLVITLYCNHRNKRGRKKLLYIFKQPFMRPVQTTQEEDGCSCRFPEEEEGGCELRVKFSRSADAPAYQQGQNQLYNELNLGRREEYDVLDKRRGRDPEMGGKPRRKNPQEGLYNELQKDKMAEAYSEIGMKGERRRGKGHDGLYQGLSTATKDTYDALHMQALPPRLCARPRRSPAQDGKVYINMPGRG

SEQ ID NO: 44 - protein, 440 aa, synthetic construct
KKVVLGKKGDTVELTCTASQKKSIQFHWKNSNQIKILGNQGSFLTKGPSKLNDRADSRRSLWDQGNFPLIIKNLKIEDSDTYICEVEDQKEEVQLLVFGLTANSDTHLLQGQSLTLTLESPPGSSPSVQCRSPRGKNIQGGKTLSVSQLELQDSGTWTCTVLQNQKKVEFKIDIVVLAAAAFVPVFLPAKPTTTPAPRPPTPAPTIASQPLSLRPEACRPAAGGAVHTRGLDFACDIYIWAPLAGTCGVLLLSLVITLYCNHRNRSKRSRLLHSDYMNMTPRRPGPTRKHYQPYAPPRDFAAYRSLCARPRRSPAQDGKVYINMPGRGRVKFSRSADAPAYQQGQNQLYNELNLGRREEYDVLDKRRGRDPEMGGKPRRKNPQEGLYNELQKDKMAEAYSEIGMKGERRRGKGHDGLYQGLSTATKDTYDALHMQALPPR

SEQ ID NO: 45 - protein, 519 aa, synthetic construct
KKVVLGKKGDTVELTCTASQKKSIQFHWKNSNQIKILGNQGSFLTKGPSKLNDRADSRRSLWDQGNFPLIIKNLKIEDSDTYICEVEDQKEEVQLLVFGLTANSDTHLLQGQSLTLTLESPPGSSPSVQCRSPRGKNIQGGKTLSVSQLELQDSGTWTCTVLQNQKKVEFKIDIVVLAAAAFVPVFLPAKPTTTPAPRPPTPAPTIASQPLSLRPEACRPAAGGAVHTRGLDFACDIYIWAPLAGTCGVLLLSLVITLYCNHRNWRRKRKEKQSETSPKEFLTIYEDVKDLKTRRNHEQEQTFPGGGSTIYSMIQSQSSAPTSQEPAYTLYSLIQPSRKSGSRKRNHSPSFNSTIYEVIGKSQPKAQNPARLSRKELENFDVYSLCARPRRSPAQDGKVYINMPGRGRVKFSRSADAPAYQQGQNQLYNELNLGRREEYDVLDKRRGRDPEMGGKPRRKNPQEGLYNELQKDKMAEAYSEIGMKGERRRGKGHDGLYQGLSTATKDTYDALHMQALPPR

SEQ ID NO: 46 - protein, 538 aa, synthetic construct
KKVVLGKKGDTVELTCTASQKKSIQFHWKNSNQIKILGNQGSFLTKGPSKLNDRADSRRSLWDQGNFPLIIKNLKIEDSDTYICEVEDQKEEVQLLVFGLTANSDTHLLQGQSLTLTLESPPGSSPSVQCRSPRGKNIQGGKTLSVSQLELQDSGTWTCTVLQNQKKVEFKIDIVVLAAAAFVPVFLPAKPTTTPAPRPPTPAPTIASQPLSLRPEACRPAAGGAVHTRGLDFACDIYIWAPLAGTCGVLLLSLVITLYCNHRNKRGRKKLLYIFKQPFMRPVQTTQEEDGCSCRFPEEEEGGCELWRRKRKEKQSETSPKEFLTIYEDVKDLKTRRNHEQEQTFPGGGSTIYSMIQSQSSAPTSQEPAYTLYSLIQPSRKSGSRKRNHSPSFNSTIYEVIGKSQPKAQNPARLSRKELENFDVYSRVKFSRSADAPAYQQGQNQLYNELNLGRREEYDVLDKRRGRDPEMGGKPRRKNPQEGLYNELQKDKMAEAYSEIGMKGERRRGKGHDGLYQGLSTATKDTYDALHMQALPPR

SEQ ID NO: 47 - protein, 19 aa, synthetic construct
ATNFSLLKQAGDVEENPGP

SEQ ID NO: 48 - protein, 224 aa, synthetic construct
ASSEDVIKEFMRFKVRMEGSVNGHEFEIEGEGEGRPYEGTQTAKLKVTKGGPLPFAWDILSPQFQYGSKAYVKHPADIPDYLKLSFPEGFKWERVMNFEDGGVVTVTQDSSLQDGEFIYKVKLRGTNFPSDGPVMQKKTMGWEASTERMYPEDGALKGEIKMRLKLKDGGHYDAEVKTTYMAKKPVQLPGAYKTDIKLDITSHNEDYTIVEQYERAEGRHSTGA

SEQ ID NO: 49 - protein, 357 aa, synthetic construct
MLLLVTSLLLCELPHPAFLLIPRKVCNGIGIGEFKDSLSINATNIKHFKNCTSISGDLHILPVAFRGDSFTHTPPLDPQELDILKTVKEITGFLLIQAWPENRTDLHAFENLEIIRGRTKQHGQFSLAVVSLNITSLGLRSLKEISDGDVIISGNKNLCYANTINWKKLFGTSGQKTKIISNRGENSCKATGQVCHALCSPEGCWGPEPRDCVSCRNVSRGRECVDKCNLLEGEPREFVENSECIQCHPECLPQAMNITCTGRGPDNCIQCAHYIDGPHCVKTCPAGVMGENNTLVWKYADAGHVCHLCHPNCTYGCTGPGLEGCPTNGPKIPSIATGMVGALLLLLVVALGIGLFM

SEQ ID NO: 50 - protein, 335 aa, synthetic construct
RKVCNGIGIGEFKDSLSINATNIKHFKNCTSISGDLHILPVAFRGDSFTHTPPLDPQELDILKTVKEITGFLLIQAWPENRTDLHAFENLEIIRGRTKQHGQFSLAVVSLNITSLGLRSLKEISDGDVIISGNKNLCYANTINWKKLFGTSGQKTKIISNRGENSCKATGQVCHALCSPEGCWGPEPRDCVSCRNVSRGRECVDKCNLLEGEPREFVENSECIQCHPECLPQAMNITCTGRGPDNCIQCAHYIDGPHCVKTCPAGVMGENNTLVWKYADAGHVCHLCHPNCTYGCTGPGLEGCPTNGPKIPSIATGMVGALLLLLVVALGIGLFM